European Patent Application EP 4 582 438 A1, published July 9, 2025. Title: 막 관통 펩타이드 도메인과 그 양 끝에 염기성 또는 극성 아미노산으로 이루어진 항균 펩타이드 및 그 변이체. Applicant: 주식회사 안단테에프엠. The sequence listing filed with the application follows.

SEQUENCE LISTING (78 sequences)

SEQ ID NO: 1 - protein, 27 aa, Homo sapiens
RHSILYGSLGSVVAGFGHFLFTSRIRR

SEQ ID NO: 2 - protein, 30 aa, Homo sapiens
RKAKEAPFVPVGIAGFAAIVAYGLYKLKSR

SEQ ID NO: 3 - protein, 40 aa, Homo sapiens
KSLSILKMVGPGFLSLGLMMLVCGLVWVPIIKKKQKHRQK

SEQ ID NO: 4 - protein, 31 aa, Homo sapiens
RKSRDSPFVPIGIAGFVTVVSCGLYKLKYRR

SEQ ID NO: 5 - protein, 25 aa, Homo sapiens
TRIAAQGFTVAAILLGLAVTAMKSR

SEQ ID NO: 6 - protein, 32 aa, Homo sapiens
RKKHRGLFLTTVAALPIWNPISEFVKWYKSHK

SEQ ID NO: 7 - protein, 27 aa, Homo sapiens
SREFLKYFGTFFGLAAISLTAGAIKKK

SEQ ID NO: 8 - protein, 26 aa, Homo sapiens
QQRAATLLLTLSNLMFLAPIAVSVRR

SEQ ID NO: 9 - protein, 27 aa, Homo sapiens
RLATRLLKLRYLILGSAVGGGYTAKKT

SEQ ID NO: 10 - protein, 27 aa, Homo sapiens
RNSAIAAGVCGALFIGYCIYFDRKRRS

SEQ ID NO: 11 - protein, 32 aa, Homo sapiens
KKNENLQNLLCGSGAGVISKTLTYPLDLFKKR

SEQ ID NO: 12 - protein, 30 aa, Homo sapiens
RWERVARYAVCAAGILLSIYAYHVEREKER

SEQ ID NO: 13 - protein, 32 aa, Homo sapiens
RRTRLILFVLLLFGIYGLLKNPFLSVRFRTTT

SEQ ID NO: 14 - protein, 30 aa, Homo sapiens
TKKDTAQIMFMAGLPIGSLIFRLITDKMGR

SEQ ID NO: 15 - protein, 25 aa, Homo sapiens
RTRLLITGLFGAGLGGAWLALRAEK

SEQ ID NO: 16 - protein, 32 aa, Homo sapiens
STRLTLLLMVATPALMGVGTLMGSGLRKLSRQ

SEQ ID NO: 17 - protein, 30 aa, Homo sapiens
RRRMKLLLGIALLAYVASVWGNFVNMRSIQ

SEQ ID NO: 18 - protein, 30 aa, Homo sapiens
RSLLRLLAAAAACGAFAFLGYCIYLNRKRR

SEQ ID NO: 19 - protein, 33 aa, Homo sapiens
KLIKTVFAFCSMLCLLNSTVNPIIYALRSKDLR

SEQ ID NO: 20 - protein, 31 aa, Homo sapiens
RKVGWVTAGLVIGAGACYCIYRLTRGRKQNK

SEQ ID NO: 21 - protein, 34 aa, Homo sapiens
KRKTFNKVLGHVNNILISAVLPTAFRVAKKRAPK

SEQ ID NO: 22 - protein, 31 aa, Homo sapiens
KKRAPKVLGTTLVVGLLAGVGYFAFMLFRKR

SEQ ID NO: 23 - protein, 33 aa, Homo sapiens
RRLSCHVLSASVGSSAVMSTAIMATLLLFKHQK

SEQ ID NO: 24 - protein, 32 aa, Homo sapiens
RILSKYHRFISFTLYLIGFCMFVLSLVKKHYR

SEQ ID NO: 25 - protein, 30 aa, Homo sapiens
RKGQERFNRWFLTGMTVAGVVLLGSLFSRK

SEQ ID NO: 26 - protein, 36 aa, Homo sapiens
KKYFNSYTLTGRMNCVLATYGSIALIVLYFKLRSKK

SEQ ID NO: 27 - protein, 29 aa, Homo sapiens
KKIFKGVLVAELVGVFGAYFLFSKMHTSQ

SEQ ID NO: 28 - protein, 31 aa, Homo sapiens
SRQNLVALTVTTLLGVAVGGFVLWKGIQRRR

SEQ ID NO: 29 - protein, 33 aa, Homo sapiens
SQIKFSPVAKKLFVVTAVSAISVIFLAHFKRKR

SEQ ID NO: 30 - protein, 31 aa, Homo sapiens
KSSTFWLRASFGATVFAVLGFAMYKALLKQR

SEQ ID NO: 31 - protein, 30 aa, Homo sapiens
RRRNQILSVLAGLAAMVGYALLSGIVSIQR

SEQ ID NO: 32 - protein, 32 aa, Homo sapiens
RRGLSGYSMLAIGIGTLIYGHWSIMKWNRERR

SEQ ID NO: 33 - protein, 28 aa, Homo sapiens
QRSRMLSIFYFAIPVGSGLGYIAGSKVK

SEQ ID NO: 34 - protein, 33 aa, Homo sapiens
KKKFYVFGVAMTMMIRVSVYPFTLIRTRLQVQK

SEQ ID NO: 35 - protein, 31 aa, Homo sapiens
KRRGGVPSLIAGLFVGCLAGYGAYRVSNDKR

SEQ ID NO: 36 - protein, 26 aa, Homo sapiens
RQKAVSLFLCYLLLFTCSGVEAGKKK

SEQ ID NO: 37 - protein, 25 aa, Homo sapiens
SILYGSLGSVVAGFGHFLFTSRIRR

SEQ ID NO: 38 - protein, 24 aa, Homo sapiens
RHSILYGSLGSVVAGFGHFLFTSR

SEQ ID NO: 39 - protein, 18 aa, synthetic construct
ILYGSLGSVVAGFGHFLF

SEQ ID NO: 40 - protein, 27 aa, Homo sapiens
KAKEAPFVPVGIAGFAAIVAYGLYKLK

SEQ ID NO: 41 - protein, 21 aa, synthetic construct
EAPFVPVGIAGFAAIVAYGLY

SEQ ID NO: 42 - protein, 23 aa, synthetic construct
KEAPFVPVGIAGFAAIVAYGLYK

SEQ ID NO: 43 - protein, 25 aa, synthetic construct
KKEAPFVPVGIAGFAAIVAYGLYKK

SEQ ID NO: 44 - protein, 27 aa, synthetic construct
KKKEAPFVPVGIAGFAAIVAYGLYKKK

SEQ ID NO: 45 - protein, 29 aa, synthetic construct
KKKKEAPFVPVGIAGFAAIVAYGLYKKKK

SEQ ID NO: 46 - protein, 31 aa, synthetic construct
KKKKKEAPFVPVGIAGFAAIVAYGLYKKKKK

SEQ ID NO: 47 - protein, 25 aa, synthetic construct
RREAPFVPVGIAGFAAIVAYGLYRR

SEQ ID NO: 48 - protein, 27 aa, synthetic construct
RRREAPFVPVGIAGFAAIVAYGLYRRR

SEQ ID NO: 49 - protein, 29 aa, synthetic construct
RRRREAPFVPVGIAGFAAIVAYGLYRRRR

SEQ ID NO: 50 - protein, 22 aa, synthetic construct
KKILYGKLGKVVAGFGHFLFKK

SEQ ID NO: 51 - protein, 24 aa, synthetic construct
KKKILYGKLGKVVAGFGHFLFKKK

SEQ ID NO: 52 - protein, 22 aa, synthetic construct
RRILYGKLGKVVAGFGHFLFRR

SEQ ID NO: 53 - protein, 24 aa, synthetic construct
RRRILYGKLGKVVAGFGHFLFRRR

SEQ ID NO: 54 - protein, 25 aa, synthetic construct
LANVIRYFPTQALNFAFKDKYKQIF

SEQ ID NO: 55 - protein, 27 aa, synthetic construct
KLANVIRYFPTQALNFAFKDKYKQIFK

SEQ ID NO: 56 - protein, 29 aa, synthetic construct
KKLANVIRYFPTQALNFAFKDKYKQIFKK

SEQ ID NO: 57 - protein, 31 aa, synthetic construct
KKKLANVIRYFPTQALNFAFKDKYKQIFKKK

SEQ ID NO: 58 - protein, 25 aa, Homo sapiens
ATVGVAGSGAGIGTVFGSLIIGYAR

SEQ ID NO: 59 - protein, 29 aa, synthetic construct
KKKKVGVAGSGAGIGTVFGSLIIGYKKKK

SEQ ID NO: 60 - protein, 24 aa, Homo sapiens
TAGLHRQLLYITAFFFAGYYLVKR

SEQ ID NO: 61 - protein, 28 aa, synthetic construct
KKKKGLHRQLLYITAFFFAGYYLVKKKK

SEQ ID NO: 62 - protein, 25 aa, Homo sapiens
HTQIAAQGFTIAAILLGLAATAMKS

SEQ ID NO: 63 - protein, 29 aa, synthetic construct
KKKKQIAAQGFTIAAILLGLAATAMKKKK

SEQ ID NO: 64 - protein, 29 aa, synthetic construct
KKKKVGPVQLAVLTCGLFLILLALHKKKK

SEQ ID NO: 65 - protein, 29 aa, synthetic construct
KKKKAATLLLTLSNLMFLAPIAVSVKKKK

SEQ ID NO: 66 - protein, 29 aa, synthetic construct
KKKKSTYMYLAGSIGLTALSAIAISKKKK

SEQ ID NO: 67 - protein, 27 aa, unidentified
RESILYGSLGSIVTGLGHFLVTSRIRR

SEQ ID NO: 68 - protein, 27 aa, unidentified
RLAARLLKLRYIILGSAVGGGYTAKKT

SEQ ID NO: 69 - protein, 31 aa, unidentified
KRKTFNKVLGHVNNILISAVLPTAFRVAKKR

SEQ ID NO: 70 - protein, 30 aa, unidentified
RKGQETFNKWLLTGATVAGVLLLGSLLSRK

SEQ ID NO: 71 - protein, 27 aa, synthetic construct
KAKIAAQGFTVAAILLGLAVTAMKKLK

SEQ ID NO: 72 - protein, 26 aa, synthetic construct
KAKGLHRQLLYITAFFFAGYYLVKLK

SEQ ID NO: 73 - protein, 21 aa, synthetic construct
VGVAGSGAGIGTVFGSLIIGY

SEQ ID NO: 74 - protein, 20 aa, synthetic construct
GLHRQLLYITAFFFAGYYLV

SEQ ID NO: 75 - protein, 21 aa, synthetic construct
QIAAQGFTIAAILLGLAATAM

SEQ ID NO: 76 - protein, 21 aa, synthetic construct
VGPVQLAVLTCGLFLILLALH

SEQ ID NO: 77 - protein, 21 aa, synthetic construct
AATLLLTLSNLMFLAPIAVSV

SEQ ID NO: 78 - protein, 21 aa, synthetic construct
STYMYLAGSIGLTALSAIAIS